European Patent Specification EP 4 011 901 B1, published August 30, 2023. Title: METHOD FOR THE FMOC GROUP CLEAVAGE. Applicant: Fresenius Kabi iPSUM Srl Alma Mater Studiorum - University of Bologna. The sequence listing filed with the application follows.

SEQUENCE LISTING (2 sequences)

SEQ ID NO: 1 - protein, 8 aa, Artificial Sequence
  Linear Octreotide
  MOD_RES (1)..(1): Xaa is D-Phe
  MOD_RES (4)..(4): Xaa is D-Trp
  MOD_RES (8)..(8): C-terminal Threoninol
XCFXKTCT

SEQ ID NO: 2 - protein, 6 aa, Artificial Sequence
  Model hexapeptide
AKDGYI